European Patent Application EP 4 692 340 A1, published February 11, 2026. Title: A novel serine protease variant. Applicant: 씨제이제일제당 주식회사. The sequence listing filed with the application follows.

SEQUENCE LISTING (32 sequences)

SEQ ID NO: 1 - DNA, 6922 bp, synthetic construct
  source 1..6922: mol_type = other DNA; note = pBE-S-TFP(F12Y/N116D)
actagtgttcttttctgtatgaaaatagttatttcgagtctctacggaaatagcgagagatgatatacctaaatagagataaaatcatctcaaaaaaatgggtctactaaaatattattccatctattacaataaattcacagaatagtcttttaagtaagtctactctgaacttaagcaaaaggagagggacgcgtgtgagaagcaaaaaattgtggatcagcttgttgtttgcgttaacgttaatctttacgatggcgttcagcaacatgtctgcgcaggctgcggccggtgcacatatgcaagagctggcgttgaaacgggacctcggcctctctgacgcagaagtagccgaactccgggctgctgaggcggaagcggtcgagctcgaggaggagctccgcgattcattagggtcagacttcggcggtgtatatctggatgctgacaccaccgaaattacggtcgcggtaaccgacccggcagcggtaagtcgtgtcgacgcggatgatgtcacagttgatgttgtcgatttcggggaaacagctttgaatgattttgtggcttcattaaatgccattgccgacacggcagaccctaaagtcactggatggtataccgatctcgaaagtgatgccgtagtcattacgaccttgcgtggcgggactcctgctgccgaggaacttgctgagagagcgggtctcgacgaaagagccgttcggattgtggaagaagatgaagaaccacagagcttggctgcaattattggtggaaacccgtactattacggaaattacagatgcagtatcgggtttagtgtccgtcagggctctcaaacgggattcgcgaccgcaggccactgcggatccacggggacgcgtgtgtcttctccttcaggaacagttgcaggaagttatttcccgggtcgcgatatgggctgggtgcggattacatcagcagatactgtaacaccactcgtaaatcggtataatgggggaactgttacggtcactgggtcacaagaagctgccaccggatcctccgtttgtcgctctggagcaacaacgggctggcgctgcggaactatccaatcaaaagaccaaacggttcgctatgcagaagggactgttactggtttaacaagaactacagcctgtgctgaaggtggggattctggagggccatggctcacaggtagccaggcgcaaggggttacaagcggcggaacaggcgattgcagaagtggagggattacctttttccaaccaatcaatccattgcttagctatttcggccttcaattagtgaccggctgaaagcttgtcgacctgcagtctagacatcaccatcatcaccactaatgcggtagtttatcacagttaaattgctaacgcagtcaggcaccgtgtatgaaatctaacaatgcgctcatcgtcatcctcggcaccgtcaccctggatgctgtaggcataggcttggttatgccggtactgccgggcctatttcactttttgcattctacaaactgcataactattatgtaaatcgctcctttttaggtggcacaaatgtgaggcattttcgctctttccggcaaccacttccaagtaaagtataacacactatactttatattcataaagtgtgtgctctgcgaggctgtcggcagtgccgaccaaaaccataaaacctttaagacctttcttttttttacgagaaaaaagaaacaaaaaaacctgccctctgccacctcagcaaaggggggttttgctctcgtgctcgtttaaaaatcagcaagggacaggtagtattttttgagaagatcactcaaaaaatctccacctttaaacccttgccaatttttattttgtccgttttgtctagcttaccgaaagccagactcagcaagaataaaatttttattgtctttcggttttctagtgtaacggacaaaaccactcaaaataaaaaagatacaagagaggtctctcgtatcttttattcagcaatcgcgcccgattgctgaacagattaataatagattttagctttttatttgttgaaaaaagctaatcaaattgttgtcgggatcaattactgcaaagtctcgttcatcccaccactgatcttttaatgatgtattggggtgcaaaatgcccaaaggcttaatatgttgatataattcatcaattccctctacttcaatgcggcaactagcagtaccagcaataaacgactccgcacctgtacaaaccggtgaatcattactacgagagcgccagccttcatcacttgcctcccatagatgaatccgaacctcattacacattagaactgcgaatccatcttcatggtgaaccaaagtgaaacctagtttatcgcaataaaaacctatactctttttaatatccccgactggcaatgccgggatagactgtaacattctcacgcataaaatcccctttcattttctaatgtaaatctattaccttattattaattcaattcgctcataattaatcctttttcttattacgcaaaatggcccgatttaagcacaccctttattccgttaatgcgccatgacagccatgataattactaatactaggagaagttaataaatacgagcaaaaggccagcaaaaggccaggaaccgtaaaaaggccgcgttgctggcgtttttccataggctccgcccccctgacgagcatcacaaaaatcgacgctcaagtcagaggtggcgaaacccgacaggactataaagataccaggcgtttccccctggaagctccctcgtgcgctctcctgttccgaccctgccgcttaccggatacctgtccgcctttctcccttcgggaagcgtggcgctttctcatagctcacgctgtaggtatctcagttcggtgtaggtcgttcgctccaagctgggctgtgtgcacgaaccccccgttcagcccgaccgctgcgccttatccggtaactatcgtcttgagtccaacccggtaagacacgacttatcgccactggcagcagccactggtaacaggattagcagagcgaggtatgtaggcggtgctacagagttcttgaagtggtggcctaactacggctacactagaagaacagtatttggtatctgcgctctgctgaagccagttaccttcggaaaaagagttggtagctcttgatccggcaaacaaaccaccgctggtagcggtggtttttttgtttgcaagcagcagattacgcgcagaaaaaaaggatctcaagaagatcctttgatcttttctacggggtctgacgctcagtggaacgaaaactcacgttaagggattttggtcatgagattatcaaaaaggatcttcacctagatccttttaaattaaaaatgaagttttaaatcaatctaaagtatatatgagtaaacttggtctgacagttaccaatgcttaatcagtgaggcacctatctcagcgatctgtctatttcgttcatccatagttgcctgactccccgtcgtgtagataactacgatacgggagggcttaccatctggccccagtgctgcaatgataccgcgagacccacgctcaccggctccagatttatcagcaataaaccagccagccggaagggccgagcgcagaagtggtcctgcaactttatccgcctccatccagtctattaattgttgccgggaagctagagtaagtagttcgccagttaatagtttgcgcaacgttgttgccattgctacaggcatcgtggtgtcacgctcgtcgtttggtatggcttcattcagctccggttcccaacgatcaaggcgagttacatgatcccccatgttgtgcaaaaaagcggttagctccttcggtcctccgatcgttgtcagaagtaagttggccgcagtgttatcactcatggttatggcagcactgcataattctcttactgtcatgccatccgtaagatgcttttctgtgactggtgagtactcaaccaagtcattctgagaatagtgtatgcggcgaccgagttgctcttgcccggcgtcaatacgggataataccgcgccacatagcagaactttaaaagtgctcatcattggaaaacgttcttcggggcgaaaactctcaaggatcttaccgctgttgagatccagttcgatgtaacccactcgtgcacccaactgatcttcagcatcttttactttcaccagcgtttctgggtgagcaaaaacaggaaggcaaaatgccgcaaaaaagggaataagggcgacacggaaatgttgaatactcatactcttcctttttcaatattattgaagcatttatcagggttattgtctcatgagcggatacatatttgaatgtatttagaaaaataaacaaataggggttccgcgcacatttccccgaaaagtgccacctgacgtctaagaaaccattattatcatgacattaacctataaaaataggcgtatcacgaggccctttcgtctcgcgcgtttcggtgatgacggtgaaaacctctgacagtaaccaacatgattaacaattattagaggtcatcgttcaaaatggtatgcgttttgacacatccactatatatccgtgtcgttctgtccactcctgaatcccattccagaaattctctagcgattccagaagtttctcagagtcggaaagttgaccagacattacgaactggcacagatggtcataacctgaaggaagatctgattgcttaactgcttcagttaagaccgaagcgctcgtcgtataacagatgcgatgatgcagaccaatcaacatggcacctgccattgctacctgtacagtcaaggatggtagaaatgttgtcggtccttgcacacgaatattacgccatttgcctgcatattcaaacagctcttctacgataagggcacaaatcgcatcgtggaacgtttgggcttctaccgatttagcagtttgatacactttctctaagtatccacctgaatcataaatcggcaaaatagagaaaaattgaccatgtgtaagcggccaatctgattccacctgagatgcataatctagtagaatctcttcgctatcaaaattcacttccaccttccactcaccggttgtccattcatggctgaactctgcttcctctgttgacatgacacacatcatctcaatatccgaatagggcccatcagtctgacgaccaagagagccataaacaccaatagccttaacatcatccccatatttatccaatattcgttccttaatttcatgaacaatcttcattctttcttctctagtcattattattggtccattcactattctcattcccttttcagataattttagatttgcttttctaaataagaatatttggagagcaccgttcttattcagctattaataactcgtcttcctaagcatccttcaatccttttaataacaattatagcatctaatcttcaacaaactggcccgtttgttgaactactctttaataaaataatttttccgttcccaattccacattgcaataatagaaaatccatcttcatcggctttttcgtcatcatctgtatgaatcaaatcgccttcttctgtgtcatcaaggtttaattttttatgtatttcttttaacaaaccaccataggagattaaccttttacggtgtaaaccttcctccaaatcagacaaacgtttcaaattcttttcttcatcatcggtcataaaatccgtatcctttacaggatattttgcagtttcgtcaattgccgattgtatatccgatttatatttatttttcggtcgaatcatttgaacttttacatttggatcatagtctaatttcattgcctttttccaaaattgaatccattgtttttgattcacgtagttttctgtattcttaaaataagttggttccacacataccaatacatgcatgtgctgattataagaattatctttattatttattgtcacttccgttgcacgcataaaaccaacaagatttttattaatttttttatattgcatcattcggcgaaatccttgagccatatctgacaaactcttatttaattcttcgccatcataaacatttttaactgttaatgtgagaaacaaccaacgaactgttggcttttgtttaataacttcagcaacaaccttttgtgactgaatgccatgtttcattgctctcctccagttgcacattggacaaagcctggatttacaaaaccacactcgatacaactttctttcgcctgtttcacgattttgtttatactctaatatttcagcacaatcttttactctttcagcctttttaaattcaagaatatgcagaagttcaaagtaatcaacattagcgattttcttttctctccatggtctcacttttccactttttgtcttgtccactaaaacccttgatttttcatctgaataaatgctactattaggacacataatattaaaagaaacccccatctatttagttatttgtttagtcacttataactttaacagatggggtttttctgtgcaaccaattttaagggttttcaatactttaaaacacatacataccaacacttcaacgcacctttcagcaactaaaataaaaatgacgttatttctatatgtatcaagataagaaagaacaagttcaaaaccatcaaaaaaagacaccttttcaggtgctttttttattttataaactcattccctgatctcgacttcgttctttttttacctctcggttatgagttagttcaaattcgttctttttaggttctaaatcgtgtttttcttggaattgtgctgttttatcctttaccttgtctacaaaccccttaaaaacgtttttaaaggcttttaagccgtctgtacgttcctaa

SEQ ID NO: 2 - DNA, 47 bp, synthetic construct
  source 1..47: mol_type = other DNA; note = TAP_mature region_F
aagaagatgaagaaccacagagcttggctgcaattattggtggaaac

SEQ ID NO: 3 - DNA, 44 bp, synthetic construct
  source 1..44: mol_type = other DNA; note = TAP_mature region_R
gactgcaggtcgacaagctttcagccggtcactaattgaaggcc

SEQ ID NO: 4 - DNA, 23 bp, synthetic construct
  source 1..23: mol_type = other DNA; note = pBE-S-vector-F
aagcttgtcgacctgcagtctag

SEQ ID NO: 5 - DNA, 24 bp, synthetic construct
  source 1..24: mol_type = other DNA; note = pBE-S-vector-R
ctgtggttcttcatcttcttccac

SEQ ID NO: 6 - protein, 338 aa, synthetic construct
  source 1..338: note = Thermobifida fusca (F163YN267D)
MQELALKRDLGLSDAEVAELRAAEAEAVELEEELRDSLGSDFGGVYLDADTTEITVAVTDPAAVSRVDADDVTVDVVDFGETALNDFVASLNAIADTADPKVTGWYTDLESDAVVITTLRGGTPAAEELAERAGLDERAVRIVEEDEEPQSLAAIIGGNPYYYGNYRCSIGFSVRQGSQTGFATAGHCGSTGTRVSSPSGTVAGSYFPGRDMGWVRITSADTVTPLVNRYNGGTVTVTGSQEAATGSSVCRSGATTGWRCGTIQSKDQTVRYAEGTVTGLTRTTACAEGGDSGGPWLTGSQAQGVTSGGTGDCRSGGITFFQPINPLLSYFGLQLVTG

SEQ ID NO: 7 - protein, 187 aa, synthetic construct
  source 1..187: note = Thermobifida fusca serine protease_mature region (F163YN267D)
LAAIIGGNPYYYGNYRCSIGFSVRQGSQTGFATAGHCGSTGTRVSSPSGTVAGSYFPGRDMGWVRITSADTVTPLVNRYNGGTVTVTGSQEAATGSSVCRSGATTGWRCGTIQSKDQTVRYAEGTVTGLTRTTACAEGGDSGGPWLTGSQAQGVTSGGTGDCRSGGITFFQPINPLLSYFGLQLVTG

SEQ ID NO: 8 - protein, 368 aa, Thermobifida fusca
  source 1..368: note = GenBank: AAZ54522.1
MNHSSRRTTSLLFTAALAATALVAATTPASAQELALKRDLGLSDAEVAELRAAKAEAVELEEELRDSLGSDFGGVYLDADTTEITVAVTDPAAVSRVDADDVTVDVVDFGETALNDFVASLNAIADTADPKVTGWYTDLESDAVVITTLRGGTPAAEELAERAGLDERAVRIVEEDEEPQSLAAIIGGNPYYFGNYRCSIGFSVRQGSQTGFATAGHCGSTGTRVSSPSGTVAGSYFPGRDMGWVRITSADTVTPLVNRYNGGTVTVTGSQEAATGSSVCRSGATTGWRCGTIQSKNQTVRYAEGTVTGLTRTTACAEGGDSGGPWLTGSQAQGVTSGGTGDCRSGGITFFQPINPLLSYFGLQLVTG

SEQ ID NO: 9 - protein, 338 aa, Thermobifida fusca
  source 1..338: note = GenBank: AAZ54522.1 derived
MQELALKRDLGLSDAEVAELRAAKAEAVELEEELRDSLGSDFGGVYLDADTTEITVAVTDPAAVSRVDADDVTVDVVDFGETALNDFVASLNAIADTADPKVTGWYTDLESDAVVITTLRGGTPAAEELAERAGLDERAVRIVEEDEEPQSLAAIIGGNPYYFGNYRCSIGFSVRQGSQTGFATAGHCGSTGTRVSSPSGTVAGSYFPGRDMGWVRITSADTVTPLVNRYNGGTVTVTGSQEAATGSSVCRSGATTGWRCGTIQSKNQTVRYAEGTVTGLTRTTACAEGGDSGGPWLTGSQAQGVTSGGTGDCRSGGITFFQPINPLLSYFGLQLVTG

SEQ ID NO: 10 - protein, 187 aa, Thermobifida fusca
  source 1..187: note = serine protease_mature region
LAAIIGGNPYYFGNYRCSIGFSVRQGSQTGFATAGHCGSTGTRVSSPSGTVAGSYFPGRDMGWVRITSADTVTPLVNRYNGGTVTVTGSQEAATGSSVCRSGATTGWRCGTIQSKNQTVRYAEGTVTGLTRTTACAEGGDSGGPWLTGSQAQGVTSGGTGDCRSGGITFFQPINPLLSYFGLQLVTG

SEQ ID NO: 11 - protein, 368 aa, Thermobifida fusca
  source 1..368: note = NCBI Accession number WP_016188200.1
MNHSSRRTTSLLFTAALAATALVAATTPASAQELALKRDLGLSDAEVAELRAAEAEAVELEEELRDSLGSDFGGVYLDADTTEITVAVTDPAAVSRVDADDVTVDVVDFGETALNDFVASLNAIADTADPKVTGWYTDLESDAVVITTLRGGTPAAEELAERAGLDERAVRIVEEDEEPQSLAAIIGGNPYYFGNYRCSIGFSVRQGSQTGFATAGHCGSTGTRVSSPSGTVAGSYFPGRDMGWVRITSADTVTPLVNRYNGGTVTVTGSQEAATGSSVCRSGATTGWRCGTIQSKNQTVRYAEGTVTGLTRTTACAEGGDSGGPWLTGSQAQGVTSGGTGDCRSGGITFFQPINPLLSYFGLQLVTG

SEQ ID NO: 12 - protein, 338 aa, Thermobifida fusca
  source 1..338: note = NCBI Accession number WP_016188200.1 derived
MQELALKRDLGLSDAEVAELRAAEAEAVELEEELRDSLGSDFGGVYLDADTTEITVAVTDPAAVSRVDADDVTVDVVDFGETALNDFVASLNAIADTADPKVTGWYTDLESDAVVITTLRGGTPAAEELAERAGLDERAVRIVEEDEEPQSLAAIIGGNPYYFGNYRCSIGFSVRQGSQTGFATAGHCGSTGTRVSSPSGTVAGSYFPGRDMGWVRITSADTVTPLVNRYNGGTVTVTGSQEAATGSSVCRSGATTGWRCGTIQSKNQTVRYAEGTVTGLTRTTACAEGGDSGGPWLTGSQAQGVTSGGTGDCRSGGITFFQPINPLLSYFGLQLVTG

SEQ ID NO: 13 - protein, 187 aa, Thermobifida halotolerans
  source 1..187: note = serine protease mature region
FTDIIGGNPYYFDGYRCSIGFSVRRGSESGFATAGHCGEEGTETSDPEGTVAGAYFPGRDMGWVRITDADTVTPLVNRYNGENVTVAGSREAATGSSVCRSGSTTGWRCGTIRSKNQTVRYIEGTVTGLTRTTACAEGGDSGGPWLTGSQGQGVTSGGSGNCTLGGVTYFQPLNPLLSHFDLDLVTG

SEQ ID NO: 14 - protein, 187 aa, Actinorugispora endophytica
  source 1..187: note = serine protease mature region
LANVIGGNAYYFGGYRCSVGFSVRHSSGPGFATAGHCGDVGTRTTSPTGTIAGSYFPGRDMGWVRITSADTVTPLVNRYNGSYITVTGSSEAANGSSVCRSGSTTGWHCGTIQSKNQTVNYAEGSVAGLTRTTACAEGGDSGGSWLTGTQAQGVTSGGSGNCTWGGTTYFQPINPLLSYFNLTLVTG

SEQ ID NO: 15 - protein, 187 aa, Thermobifida cellulosilytica
  source 1..187: note = serine protease mature region
FADVIGGNPYYFGGYRCSIGFSVRKGSDTGFATAGHCGETGTLTRSPEGVVAGSYFPGRDMGWVRLTGADTVTPLVNRYDGGTVTVTGSQEAVTGSSVCRSGSTTGWRCGIIQSKNQTVRYAEGTVTGLTRTTACAEAGDSGGPWLTGSQAQGVTSGGSGNCRTGGITYFQPINPLLSYFGLELVTG

SEQ ID NO: 16 - DNA, 1107 bp, Thermobifida fusca
  source 1..1107: mol_type = genomic DNA; note = encoding GenBank: AAZ54522.1
gtgaaccattcctcccgaagaaccacctccctccttttcactgccgcgctggccgccactgcactggtcgccgccaccacccccgcctccgcccaagagctcgccctcaaacgcgacctcgggttgagcgacgctgaagtcgcggaactgcgcgccgccaaagccgaagcagtcgagctggaagaggagctgcgcgactccctcggctccgatttcggcggcgtctacttggacgcggacaccacagagatcacggtcgccgtcaccgaccccgccgccgtgtcccgtgtcgacgcggacgacgtcaccgtggacgttgttgatttcggggaaaccgccctcaacgacttcgtggcgtccctcaacgcgatcgctgacaccgctgacccaaaggtcaccggctggtacaccgacctggagtccgatgcggtagtcatcaccacgctccggggcggcactccggcagccgaagagctcgccgagcgggctggtctggacgagcgggccgtgcgcattgtcgaagaggacgaagagccgcagtcccttgccgccatcatcggcggcaacccctactatttcgggaactaccgctgctctatcggattctcggtccgccagggcagccagaccggcttcgccaccgcgggccactgcggttcgacaggcacgcgagtcagctccccctcaggcactgtcgccggatcgtacttccccggccgtgacatgggctgggtgcgtatcaccagcgctgacaccgtcaccccgctcgtcaaccgctacaacggcggaacggtgaccgtcaccggttcgcaggaggccgccaccggctcttcggtgtgccgctccggagcgaccaccgggtggcgctgcggcaccatccagtcgaagaaccagaccgtccgctacgcggaaggaaccgtcaccggcctgacccgcaccactgcctgcgctgaaggcggcgactccggcggcccgtggctcaccggttcccaagcccaaggggtgacctcgggcggcaccggtgactgccggtccggcggcatcacgttcttccagcccatcaacccgctgctgtcctacttcggactgcaactggtcaccggctga

SEQ ID NO: 17 - DNA, 46 bp, synthetic construct
  source 1..46: mol_type = other DNA; note = F331Y F
ccaaccaatcaatccattgcttagctattacggccttcaattagtg

SEQ ID NO: 18 - DNA, 46 bp, synthetic construct
  source 1..46: mol_type = other DNA; note = F331Y R
cactaattgaaggccgtaatagctaagcaatggattgattggttgg

SEQ ID NO: 19 - DNA, 48 bp, synthetic construct
  source 1..48: mol_type = other DNA; note = F331E F
ccaaccaatcaatccattgcttagctatgagggccttcaattagtgac

SEQ ID NO: 20 - DNA, 48 bp, synthetic construct
  source 1..48: mol_type = other DNA; note = F331E R
gtcactaattgaaggccctcatagctaagcaatggattgattggttgg

SEQ ID NO: 21 - DNA, 46 bp, synthetic construct
  source 1..46: mol_type = other DNA; note = F331H F
tccaaccaatcaatccattgcttagctatcacggccttcaattagt

SEQ ID NO: 22 - DNA, 46 bp, synthetic construct
  source 1..46: mol_type = other DNA; note = F331H R
actaattgaaggccgtgatagctaagcaatggattgattggttgga

SEQ ID NO: 23 - DNA, 45 bp, synthetic construct
  source 1..45: mol_type = other DNA; note = F331L F
caaccaatcaatccattgcttagctatttaggccttcaattagtg

SEQ ID NO: 24 - DNA, 45 bp, synthetic construct
  source 1..45: mol_type = other DNA; note = F331L R
cactaattgaaggcctaaatagctaagcaatggattgattggttg

SEQ ID NO: 25 - DNA, 46 bp, synthetic construct
  source 1..46: mol_type = other DNA; note = F331M F
caaccaatcaatccattgcttagctatatgggccttcaattagtga

SEQ ID NO: 26 - DNA, 46 bp, synthetic construct
  source 1..46: mol_type = other DNA; note = F331M R
tcactaattgaaggcccatatagctaagcaatggattgattggttg

SEQ ID NO: 27 - DNA, 46 bp, synthetic construct
  source 1..46: mol_type = other DNA; note = F331N F
tccaaccaatcaatccattgcttagctataacggccttcaattagt

SEQ ID NO: 28 - DNA, 46 bp, synthetic construct
  source 1..46: mol_type = other DNA; note = F331N R
actaattgaaggccgttatagctaagcaatggattgattggttgga

SEQ ID NO: 29 - DNA, 48 bp, synthetic construct
  source 1..48: mol_type = other DNA
ccaaccaatcaatccattgcttagctatcagggccttcaattagtgac

SEQ ID NO: 30 - DNA, 48 bp, synthetic construct
  source 1..48: mol_type = other DNA; note = F331Q R
gtcactaattgaaggccctgatagctaagcaatggattgattggttgg

SEQ ID NO: 31 - DNA, 46 bp, synthetic construct
  source 1..46: mol_type = other DNA; note = F331W F
ccaaccaatcaatccattgcttagctattggggccttcaattagtg

SEQ ID NO: 32 - DNA, 46 bp, synthetic construct
  source 1..46: mol_type = other DNA; note = F331W R
cactaattgaaggccccaatagctaagcaatggattgattggttgg